European Patent Application EP 4 620 969 A1, published September 24, 2025. Title: Peptide Having Activity of Skin Whitening and Uses Thereof. Applicant: CAREGEN CO., LTD. The sequence listing filed with the application follows.

SEQUENCE LISTING (9 sequences)

SEQ ID NO: 1 - protein, 5 aa, synthetic construct
MLKML

SEQ ID NO: 2 - DNA, 20 bp, synthetic construct
  source 1..20: mol_type = other DNA
tgctagcagcctctctctcc

SEQ ID NO: 3 - DNA, 20 bp, synthetic construct
  source 1..20: mol_type = other DNA
cttcaaggggaaccagatga

SEQ ID NO: 4 - DNA, 20 bp, synthetic construct
  source 1..20: mol_type = other DNA
ggagccaaaagggtcatcat

SEQ ID NO: 5 - DNA, 20 bp, synthetic construct
  source 1..20: mol_type = other DNA
gtgatggcatggactgtggt

SEQ ID NO: 6 - DNA, 20 bp, synthetic construct
  source 1..20: mol_type = other DNA
gccgtctatttgccacacac

SEQ ID NO: 7 - DNA, 20 bp, synthetic construct
  source 1..20: mol_type = other DNA
gcagtcagcaacttcatggc

SEQ ID NO: 8 - DNA, 20 bp, synthetic construct
  source 1..20: mol_type = other DNA
tgaccaaacgtatccccctg

SEQ ID NO: 9 - DNA, 20 bp, synthetic construct
  source 1..20: mol_type = other DNA
ggtgtctgccgttgaagaga